European Patent Application EP 4 428 145 A1, published September 11, 2024. Title: Antimicrobial peptide. Applicant: 住友化学株式会社. Application EP 22 889 956.3, filed November 1, 2022. The sequence listing filed with the application follows.

SEQUENCE LISTING (9 sequences)

SEQ ID NO: 1 - protein, 64 aa, Lactobacillus sp. SC-2001
MASLTSFSNISEDVLSKVKGGKIIRISKWSYYNTKTKKYYADNSAIMSTLGHTVVNGWVEHFPY

SEQ ID NO: 2 - DNA, 195 bp, Lactobacillus sp. SC-2001
  source 1..195: mol_type = genomic DNA
atggcaagtttaactagtttttctaatatttctgaggatgttctttcaaaagttaaaggtggaaagattatccgtatttcaaaatggagttactataacacaaagacaaaaaaatactatgcagataattctgctattatgtctactctagggcatactgttgtcaatggctgggttgaacacttcccatattaa

SEQ ID NO: 3 - protein, 43 aa, Lactobacillus sp. SC-2001
KIIRISKWSYYNTKTKKYYADNSAIMSTLGHTVVNGWVEHFPY

SEQ ID NO: 4 - protein, 17 aa, Lactobacillus sp. SC-2001
KIIRISKWSYYNTKTKK

SEQ ID NO: 5 - protein, 26 aa, Lactobacillus sp. SC-2001
YYADNSAIMSTLGHTVVNGWVEHFPY

SEQ ID NO: 6 - protein, 9 aa, Lactobacillus sp. SC-2001
KIIRISKWS

SEQ ID NO: 7 - protein, 34 aa, Lactobacillus sp. SC-2001
YYNTKTKKYYADNSAIMSTLGHTVVNGWVEHFPY

SEQ ID NO: 8 - protein, 54 aa, Lactococcus lactis subsp. lactis
KLTFIQSTAAGDLYYNTNTHKYVYQQTQNAFGAAANTIVNGWMGGAAGGFGLHH

SEQ ID NO: 9 - protein, 64 aa, Lactobacillus johnsonii
MSKFQQLTPEDLMETKGGKIYHATPWQICNSKTHKCWADNAAIARTCGRVIVNGWLQHGPWGAR